European Patent Application EP 4 197 544 A1, published June 21, 2023. Title: METHODS FOR TREATING HEPATITIS B INFECTION. Applicant: Dicerna Pharmaceuticals, Inc. The sequence listing filed with the application follows.

SEQUENCE LISTING (65 sequences)

SEQ ID NO: 1 - RNA, 18 nt, synthetic construct
  misc_feature 1..18: note = Synthetic Polynucleotide
  misc_feature 5: note = n is a, c, g, or u
  source 1..18: mol_type = other RNA
acaanaatcctcacaata

SEQ ID NO: 2 - RNA, 15 nt, synthetic construct
  misc_feature 1..15: note = Synthetic Polynucleotide
  misc_feature 3: note = n is a, c, g, or u
  misc_feature 15: note = n is a, c, g, or u
  source 1..15: mol_type = other RNA
ttnttgtgaggattn

SEQ ID NO: 3 - RNA, 20 nt, synthetic construct
  misc_feature 1..20: note = Synthetic Polynucleotide
  misc_feature 15: note = n is a, c, g, or u
  source 1..20: mol_type = other RNA
ttattgtgaggattnttgtc

SEQ ID NO: 4 - RNA, 22 nt, synthetic construct
  misc_feature 1..22: note = Synthetic Polynucleotide
  misc_feature 15: note = n is a, c, g, or u
  source 1..22: mol_type = other RNA
ttattgtgaggattnttgtcgg

SEQ ID NO: 5 - RNA, 22 nt, synthetic construct
  misc_feature 1..22: note = Synthetic Polynucleotide
  source 1..22: mol_type = other RNA
ttattgtgaggattcttgtcgg

SEQ ID NO: 6 - RNA, 22 nt, synthetic construct
  misc_feature 1..22: note = Synthetic Polynucleotide
  source 1..22: mol_type = other RNA
ttattgtgaggatttttgtcgg

SEQ ID NO: 7 - RNA, 19 nt, synthetic construct
  misc_feature 1..19: note = Synthetic Polynucleotide
  misc_feature 5: note = n is a, c, g, or u
  source 1..19: mol_type = other RNA
acaanaatcctcacaataa

SEQ ID NO: 8 - RNA, 36 nt, synthetic construct
  misc_feature 1..36: note = Synthetic Polynucleotide
  misc_feature 6: note = n is a, c, g, or u
  source 1..36: mol_type = other RNA
gacaanaatcctcacaataagcagccgaaaggctgc

SEQ ID NO: 9 - RNA, 36 nt, synthetic construct
  misc_feature 1..36: note = Synthetic Polynucleotide
  source 1..36: mol_type = other RNA
gacaaaaatcctcacaataagcagccgaaaggctgc

SEQ ID NO: 10 - RNA, 36 nt, synthetic construct
  misc_feature 1..36: note = Synthetic Polynucleotide
  source 1..36: mol_type = other RNA
gacaagaatcctcacaataagcagccgaaaggctgc

SEQ ID NO: 11 - DNA, 10 bp, synthetic construct
  misc_feature 1..10: note = Synthetic Polynucleotide
  source 1..10: mol_type = other DNA
aatcctcaca

SEQ ID NO: 12 - RNA, 10 nt, synthetic construct
  misc_feature 1..10: note = Synthetic Polynucleotide
  source 1..10: mol_type = other RNA
tgtgaggatt

SEQ ID NO: 13 - DNA, 10 bp, synthetic construct
  misc_feature 1..10: note = Synthetic Polynucleotide
  source 1..10: mol_type = other DNA
tgtgaggatt

SEQ ID NO: 14 - DNA, 20 bp, synthetic construct
  misc_feature 1..20: note = Synthetic Polynucleotide
  source 1..20: mol_type = other DNA
tattgtgaggattcttgtca

SEQ ID NO: 15 - DNA, 20 bp, synthetic construct
  misc_feature 1..20: note = Synthetic Polynucleotide
  source 1..20: mol_type = other DNA
cggtattgtgaggattcttg

SEQ ID NO: 16 - DNA, 20 bp, synthetic construct
  misc_feature 1..20: note = Synthetic Polynucleotide
  source 1..20: mol_type = other DNA
tgtgaggattcttgtcaaca

SEQ ID NO: 17 - RNA, 21 nt, synthetic construct
  misc_feature 1..21: note = Synthetic Polynucleotide
  source 1..21: mol_type = other RNA
tattgtgaggatttttgtcaa

SEQ ID NO: 18 - DNA, 21 bp, synthetic construct
  misc_feature 1..21: note = Synthetic Polynucleotide
  source 1..21: mol_type = other DNA
  misc_feature 1..19: note = RNA
tgcggtattgtgaggattctt

SEQ ID NO: 19 - DNA, 23 bp, synthetic construct
  misc_feature 1..23: note = Synthetic Polynucleotide
  source 1..23: mol_type = other DNA
acagcattgtgaggattcttgtc

SEQ ID NO: 20 - RNA, 23 nt, synthetic construct
  misc_feature 1..23: note = Synthetic Polynucleotide
  source 1..23: mol_type = other RNA
tattgtgaggatttttgtcaaca

SEQ ID NO: 21 - RNA, 23 nt, synthetic construct
  misc_feature 1..23: note = Synthetic Polynucleotide
  source 1..23: mol_type = other RNA
attgtgaggatttttgtcaacaa

SEQ ID NO: 22 - RNA, 23 nt, synthetic construct
  misc_feature 1..23: note = Synthetic Polynucleotide
  source 1..23: mol_type = other RNA
ttgtgaggatttttgtcaacaag

SEQ ID NO: 23 - RNA, 36 nt, synthetic construct
  misc_feature 1..36: note = Synthetic Polynucleotide
  source 1..36: mol_type = other RNA
gtggtggacttctctcaatagcagccgaaaggctgc

SEQ ID NO: 24 - RNA, 22 nt, synthetic construct
  misc_feature 1..22: note = Synthetic Polynucleotide
  source 1..22: mol_type = other RNA
tattgagagaagtccaccacgg

SEQ ID NO: 25 - RNA, 22 nt, synthetic construct
  misc_feature 1..22: note = Synthetic Polynucleotide
  source 1..22: mol_type = other RNA
tttgtgaggatttttgtcaagg

SEQ ID NO: 26 - RNA, 22 nt, synthetic construct
  misc_feature 1..22: note = Synthetic Polynucleotide
  source 1..22: mol_type = other RNA
tctgagagaagtccaccacggg

SEQ ID NO: 27 - RNA, 22 nt, synthetic construct
  misc_feature 1..22: note = Synthetic Polynucleotide
  source 1..22: mol_type = other RNA
tactgagagaagtccaccacgg

SEQ ID NO: 28 - RNA, 22 nt, synthetic construct
  misc_feature 1..22: note = Synthetic Polynucleotide
  source 1..22: mol_type = other RNA
taaaactgagagaagtccacgg

SEQ ID NO: 29 - DNA, 19 bp, synthetic construct
  misc_feature 1..19: note = Synthetic Polynucleotide
  source 1..19: mol_type = other DNA
gacaagaatcctcacaata

SEQ ID NO: 30 - DNA, 19 bp, synthetic construct
  misc_feature 1..19: note = Synthetic Polynucleotide
  source 1..19: mol_type = other DNA
cgtggtggacttctctcaa

SEQ ID NO: 31 - DNA, 19 bp, synthetic construct
  misc_feature 1..19: note = Synthetic Polynucleotide
  source 1..19: mol_type = other DNA
gtggacttctctcaatttt

SEQ ID NO: 32 - DNA, 19 bp, synthetic construct
  misc_feature 1..19: note = Synthetic Polynucleotide
  misc_feature 6: note = n is a, c, g, or t
  source 1..19: mol_type = other DNA
gacaanaatcctcacaata

SEQ ID NO: 33 - DNA, 19 bp, synthetic construct
  misc_feature 1..19: note = Synthetic Polynucleotide
  misc_feature 19: note = n is a, c, g, or t
  source 1..19: mol_type = other DNA
cgtggtggacttctctcan

SEQ ID NO: 34 - DNA, 19 bp, synthetic construct
  misc_feature 1..19: note = Synthetic Polynucleotide
  misc_feature 15: note = n is a, c, g, or t
  source 1..19: mol_type = other DNA
gtggacttctctcantttt

SEQ ID NO: 35 - DNA, 22 bp, synthetic construct
  misc_feature 1..22: note = Synthetic Polynucleotide
  source 1..22: mol_type = other DNA
tgttgacaagaatcctcacaat

SEQ ID NO: 36 - DNA, 21 bp, synthetic construct
  misc_feature 1..21: note = Synthetic Polynucleotide
  source 1..21: mol_type = other DNA
tcgtggtggacttctctcaat

SEQ ID NO: 37 - DNA, 22 bp, synthetic construct
  misc_feature 1..22: note = Synthetic Polynucleotide
  misc_feature 10: note = n is a, c, g, or t
  source 1..22: mol_type = other DNA
tgttgacaanaatcctcacaat

SEQ ID NO: 38 - DNA, 21 bp, synthetic construct
  misc_feature 1..21: note = Synthetic Polynucleotide
  misc_feature 20: note = n is a, c, g, or t
  source 1..21: mol_type = other DNA
tcgtggtggacttctctcant

SEQ ID NO: 39 - RNA, 36 nt, synthetic construct
  misc_feature 1..36: note = Synthetic Polynucleotide
  source 1..36: mol_type = other RNA
tgcacttcgcgtcacctctagcagccgaaaggctgc

SEQ ID NO: 40 - RNA, 22 nt, synthetic construct
  misc_feature 1..22: note = Synthetic Polynucleotide
  source 1..22: mol_type = other RNA
tagaggtgacgcgaagtgcagg

SEQ ID NO: 41 - RNA, 36 nt, synthetic construct
  misc_feature 1..36: note = Synthetic Polynucleotide
  source 1..36: mol_type = other RNA
gcacctctctttacgcggaagcagccgaaaggctgc

SEQ ID NO: 42 - RNA, 22 nt, synthetic construct
  misc_feature 1..22: note = Synthetic Polynucleotide
  source 1..22: mol_type = other RNA
ttccgcgtaaagagaggtgcgg

SEQ ID NO: 43 - RNA, 36 nt, synthetic construct; identical to SEQ ID NO: 9
  misc_feature 1..36: note = Synthetic Polynucleotide
  misc_feature 1: note = may be modified by 2'-O-methyl ribonucleotide
  misc_feature 1..2: note = may be modified by phosphorothioate
  misc_feature 2: note = may be modified by 2'-O-methyl ribonucleotide
  misc_feature 3: note = may be modified by 2'-fluoro-deoxyribonucleotide
  misc_feature 4..7: note = may be modified by 2'-O-methyl ribonucleotide
  misc_feature 8..10: note = may be modified by 2'-fluoro-deoxyribonucleotide
  misc_feature 11: note = may be modified by 2'-O-methyl ribonucleotide
  misc_feature 12..13: note = may be modified by 2'-fluoro-deoxyribonucleotide
  misc_feature 14..16: note = may be modified by 2'-O-methyl ribonucleotide
  misc_feature 17: note = may be modified by 2'-fluoro-deoxyribonucleotide
  misc_feature 18..26: note = may be modified by 2'-O-methyl ribonucleotide
  misc_feature 27: note = may be modified by 2'-modified-GalNAc guanosine
  misc_feature 28..30: note = may be modified by 2'-modified-GalNAc adenosine
  misc_feature 31..36: note = may be modified by 2'-O-methyl ribonucleotide
  source 1..36: mol_type = other RNA

SEQ ID NO: 44 - RNA, 22 nt, synthetic construct
  misc_feature 1..22: note = Synthetic Polynucleotide
  misc_feature 1: note = may be modified by 4'-O-monomethylphosphonate-2'-O-methyl uridine
  misc_feature 1..4: note = may be modified by phosphorothioate
  misc_feature 2..3: note = may be modified by 2'-fluoro-deoxyribonucleotide
  misc_feature 4: note = may be modified by 2'-O-methyl ribonucleotide
  misc_feature 5: note = may be modified by 2'-fluoro-deoxyribonucleotide
  misc_feature 6: note = may be modified by 2'-O-methyl ribonucleotide
  misc_feature 7..8: note = may be modified by 2'-fluoro-deoxyribonucleotide
  misc_feature 9: note = may be modified by 2'-O-methyl ribonucleotide
  misc_feature 10: note = may be modified by 2'-fluoro-deoxyribonucleotide
  misc_feature 11: note = may be modified by 2'-O-methyl ribonucleotide
  misc_feature 12: note = may be modified by 2'-fluoro-deoxyribonucleotide
  misc_feature 13: note = may be modified by 2'-O-methyl ribonucleotide
  misc_feature 14: note = may be modified by 2'-fluoro-deoxyribonucleotide
  misc_feature 15: note = may be modified by 2'-O-methyl ribonucleotide
  misc_feature 16: note = may be modified by 2'-fluoro-deoxyribonucleotide
  misc_feature 17..18: note = may be modified by 2'-O-methyl ribonucleotide
  misc_feature 19: note = may be modified by 2'-fluoro-deoxyribonucleotide
  misc_feature 20..22: note = may be modified by 2'-O-methyl ribonucleotide
  misc_feature 20..22: note = may be modified by phosphorothioate
  source 1..22: mol_type = other RNA
ttattgtgaggatttttgtcgg

SEQ ID NO: 45 - DNA, 50 bp, synthetic construct
  misc_feature 1..50: note = Synthetic Polynucleotide
  source 1..50: mol_type = other DNA
tgttgacaagaatcctcacaatacctcgtggtggacttctctcaattttc

SEQ ID NO: 46 - RNA, 22 nt, synthetic construct
  misc_feature 1..22: note = Synthetic Polynucleotide
  source 1..22: mol_type = other RNA
ggaactgtttttaggagtgttt

SEQ ID NO: 47 - RNA, 22 nt, synthetic construct
  misc_feature 1..22: note = Synthetic Polynucleotide
  source 1..22: mol_type = other RNA
ggaactgttcttaggagtgttt

SEQ ID NO: 48 - RNA, 22 nt, synthetic construct
  misc_feature 1..22: note = Synthetic Polynucleotide
  source 1..22: mol_type = other RNA
ggctgtttttaggagtgttatt

SEQ ID NO: 49 - RNA, 22 nt, synthetic construct
  misc_feature 1..22: note = Synthetic Polynucleotide
  source 1..22: mol_type = other RNA
ggctgttcttaggagtgttatt

SEQ ID NO: 50 - DNA, 22 bp, synthetic construct
  misc_feature 1..22: note = Synthetic Polynucleotide
  source 1..22: mol_type = other DNA
ttgacaagaatcctcacaatac

SEQ ID NO: 51 - RNA, 22 nt, synthetic construct
  misc_feature 1..22: note = Synthetic Polynucleotide
  source 1..22: mol_type = other RNA
gggcaccacctgaagagagtct

SEQ ID NO: 52 - RNA, 22 nt, synthetic construct
  misc_feature 1..22: note = Synthetic Polynucleotide
  source 1..22: mol_type = other RNA
gggcaccacctgaagagagttt

SEQ ID NO: 53 - DNA, 22 bp, synthetic construct
  misc_feature 1..22: note = Synthetic Polynucleotide
  source 1..22: mol_type = other DNA
ctcgtggtggacttctctcaat

SEQ ID NO: 54 - RNA, 22 nt, synthetic construct
  misc_feature 1..22: note = Synthetic Polynucleotide
  source 1..22: mol_type = other RNA
ggcaccacctgaagagagtcat

SEQ ID NO: 55 - RNA, 22 nt, synthetic construct
  misc_feature 1..22: note = Synthetic Polynucleotide
  source 1..22: mol_type = other RNA
ggcaccacctgaagagagttat

SEQ ID NO: 56 - DNA, 22 bp, synthetic construct
  misc_feature 1..22: note = Synthetic Polynucleotide
  source 1..22: mol_type = other DNA
tcgtggtggacttctctcaatt

SEQ ID NO: 57 - RNA, 22 nt, synthetic construct
  misc_feature 1..22: note = Synthetic Polynucleotide
  source 1..22: mol_type = other RNA
ggcacctgaagagagtcaaaat

SEQ ID NO: 58 - RNA, 22 nt, synthetic construct
  misc_feature 1..22: note = Synthetic Polynucleotide
  source 1..22: mol_type = other RNA
ggcacctgaagagagttaaaat

SEQ ID NO: 59 - DNA, 22 bp, synthetic construct
  misc_feature 1..22: note = Synthetic Polynucleotide
  source 1..22: mol_type = other DNA
tggtggacttctctcaattttc

SEQ ID NO: 60 - RNA, 22 nt, synthetic construct
  misc_feature 1..22: note = Synthetic Polynucleotide
  source 1..22: mol_type = other RNA
tttgtgaggattcttgtcaagg

SEQ ID NO: 61 - RNA, 22 nt, synthetic construct
  misc_feature 1..22: note = Synthetic Polynucleotide
  source 1..22: mol_type = other RNA
tttgagagaagtccaccacggg

SEQ ID NO: 62 - RNA, 22 nt, synthetic construct
  misc_feature 1..22: note = Synthetic Polynucleotide
  source 1..22: mol_type = other RNA
tattgagagaagtccaccacgg

SEQ ID NO: 63 - RNA, 22 nt, synthetic construct
  misc_feature 1..22: note = Artificial Sequence
  source 1..22: mol_type = other RNA
taaaattgagagaagtccacgg

SEQ ID NO: 64 - DNA, 24 bp, synthetic construct
  misc_feature 1..24: note = Synthetic Polynucleotide
  source 1..24: mol_type = other DNA
tgttgacaagaatcctcacaatac

SEQ ID NO: 65 - DNA, 26 bp, synthetic construct
  misc_feature 1..26: note = Synthetic Polynucleotide
  source 1..26: mol_type = other DNA
ctcgtggtggacttctctcaattttc